European Patent Application EP 4 197 552 A1, published June 21, 2023. Title: METHODS AND COMPOSITIONS FOR USE OF TUMOR SELF-ANTIGENS IN ADOPTIVE IMMUNOTHERAPY. Applicant: The Children's Hospital of Philadelphia. Application EP 19767951.7, filed October 12, 2020. The sequence listing filed with the application follows.

SEQUENCE LISTING (164 sequences)

SEQ ID NO: 1 - protein, 10 aa, Homo sapiens
LLPLLPPLSP

SEQ ID NO: 2 - protein, 10 aa, Zea mays
FLDETLRSLA

SEQ ID NO: 3 - protein, 9 aa, Homo sapiens
QYNPIRTTF

SEQ ID NO: 4 - protein, 9 aa, Homo sapiens
SYQKVIELF

SEQ ID NO: 5 - protein, 9 aa, Homo sapiens
IYPDITYSL

SEQ ID NO: 6 - protein, 9 aa, Homo sapiens
FLIENLLAA

SEQ ID NO: 7 - protein, 9 aa, Homo sapiens
ALLSGVRQV

SEQ ID NO: 8 - protein, 11 aa, Homo sapiens
VLFENTDSVHL

SEQ ID NO: 9 - protein, 9 aa, Homo sapiens
SAAMVFSAL

SEQ ID NO: 10 - protein, 21 aa, synthetic construct
  REGION 1..21: note = Synthetic peptide
IYIWAPLAGTCGVLLLSLVIT

SEQ ID NO: 11 - DNA, 63 bp, synthetic construct
  misc_feature 1..63: note = Synthetic primer
  source 1..63: mol_type = other DNA
atctacatctgggctccactggcaggaacctgtggcgtgctgctgctgtccctggtcatcaca

SEQ ID NO: 12 - protein, 27 aa, synthetic construct
  REGION 1..27: note = Synthetic peptide
FWVLVVVGGVLACYSLLVTVAFIIFWV

SEQ ID NO: 13 - DNA, 81 bp, synthetic construct
  misc_feature 1..81: note = Synthetic peptide
  source 1..81: mol_type = other DNA
ttttgggtgctggtggtggttggtggagtcctggcttgctatagcttgctagtaacagtggcctttattattttctgggtg

SEQ ID NO: 14 - DNA, 339 bp, synthetic construct
  misc_feature 1..339: note = Synthetic primer
  source 1..339: mol_type = other DNA
agagtgaagttcagcaggagcgcagacgcccccgcgtaccagcagggccagaaccagctctataacgagctcaatctaggacgaagagaggagtacgatgttttggacaagagacgtggccgggaccctgagatggggggaaagccgagaaggaagaaccctcaggaaggcctgtacaatgaactgcagaaagataagatggcggaggcctacagtgagattgggatgaaaggcgagcgccggaggggcaaggggcacgatggcctttaccagggtctcagtacagccaccaaggacacctacgacgcccttcacatgcaggccctgccccctcgctaa

SEQ ID NO: 15 - protein, 41 aa, synthetic construct
  REGION 1..41: note = Synthetic peptide
RSKRSRLLHSDYMNMTPRRPGPTRKHYQPYAPPRDFAAYRS

SEQ ID NO: 16 - DNA, 123 bp, synthetic construct
  misc_feature 1..123: note = Synthetic peptide
  source 1..123: mol_type = other DNA
aggagtaagaggagcaggctcctgcacagtgactacatgaacatgactccccgccgccccgggcccacccgcaagcattaccagccctatgccccaccacgcgacttcgcagcctatcgctcc

SEQ ID NO: 17 - protein, 42 aa, synthetic construct
  REGION 1..42: note = Synthetic peptide
KRGRKKLLYIFKQPFMRPVQTTQEEDGCSCRFPEEEEGGCEL

SEQ ID NO: 18 - DNA, 126 bp, synthetic construct
  misc_feature 1..126: note = Synthetic primer
  source 1..126: mol_type = other DNA
aaacggggcagaaagaaactcctgtatatattcaaacaaccatttatgagaccagtacaaactactcaagaggaagatggctgtagctgccgatttccagaagaagaagaaggaggatgtgaactg

SEQ ID NO: 19 - protein, 15 aa, synthetic construct
  REGION 1..15: note = Synthetic peptide
GGGGSGGGGSGGGGS

SEQ ID NO: 20 - DNA, 63 bp, synthetic construct
  misc_feature 1..63: note = Synthetic primer
  source 1..63: mol_type = other DNA
atggccttaccagtgaccgccttgctcctgccgctggccttgctgctccacgccgccaggccg

SEQ ID NO: 21 - DNA, 45 bp, synthetic construct
  misc_feature 1..45: note = Synthetic primer
  source 1..45: mol_type = other DNA
ggtggaggcggttcaggtggcggcggttcgggcggtggcggctct

SEQ ID NO: 22 - DNA, 135 bp, synthetic construct
  misc_feature 1..135: note = Synthetic primer
  source 1..135: mol_type = other DNA
accacgacgccagcgccgcgaccaccaacaccggcgcccaccatcgcgtcgcagcccctgtccctgcgcccagaggcgtgccggccagcggcggggggcgcagtgcacacgagggggctggacttcgcctgtgat

SEQ ID NO: 23 - protein, 9 aa, Homo sapiens
LLLPLLPPL

SEQ ID NO: 24 - protein, 12 aa, Homo sapiens
LLLPLLPPLSPS

SEQ ID NO: 25 - protein, 9 aa, synthetic construct
  REGION 1..9: note = Synthetic peptide
TVRPKNAAL

SEQ ID NO: 26 - protein, 9 aa, synthetic construct
  REGION 1..9: note = Synthetic peptide
KATEYVHSL

SEQ ID NO: 27 - protein, 17 aa, synthetic construct
  REGION 1..17: note = Synthetic peptide
LERQRRNDLRSSFLTLR

SEQ ID NO: 28 - protein, 33 aa, synthetic construct
  REGION 1..33: note = Synthetic peptide
TVRPKNAALGPGRAQSSELILKRCLPIHQQHNY

SEQ ID NO: 29 - protein, 11 aa, synthetic construct
  REGION 1..11: note = Synthetic peptide
YPSKPDNPGED

SEQ ID NO: 30 - protein, 9 aa, synthetic construct
  REGION 1..9: note = Synthetic peptide
RYYSALRHY

SEQ ID NO: 31 - protein, 11 aa, synthetic construct
  REGION 1..11: note = Synthetic peptide
SPETLISDLLM

SEQ ID NO: 32 - protein, 8 aa, synthetic construct
  REGION 1..8: note = Synthetic peptide
TLISDLLM

SEQ ID NO: 33 - protein, 11 aa, synthetic construct
  REGION 1..11: note = Synthetic peptide
SSPETLISDLL

SEQ ID NO: 34 - protein, 9 aa, synthetic construct
  REGION 1..9: note = Synthetic peptide
SALRHYINL

SEQ ID NO: 35 - protein, 10 aa, synthetic construct
  REGION 1..10: note = Synthetic peptide
SSPETLISDL

SEQ ID NO: 36 - protein, 10 aa, synthetic construct
  REGION 1..10: note = Synthetic peptide
SPETLISDLL

SEQ ID NO: 37 - protein, 10 aa, synthetic construct
  REGION 1..10: note = Synthetic peptide
YPSKPDNPGE

SEQ ID NO: 38 - protein, 12 aa, synthetic construct
  REGION 1..12: note = Synthetic peptide
YPSKPDNPGEDA

SEQ ID NO: 39 - protein, 8 aa, synthetic construct
  REGION 1..8: note = Synthetic peptide
STENVPRT

SEQ ID NO: 40 - protein, 8 aa, synthetic construct
  REGION 1..8: note = Synthetic peptide
TENVPRTR

SEQ ID NO: 41 - protein, 10 aa, synthetic construct
  REGION 1..10: note = Synthetic peptide
RESTENVPRT

SEQ ID NO: 42 - protein, 9 aa, synthetic construct
  REGION 1..9: note = Synthetic peptide
YPSKPDNPG

SEQ ID NO: 43 - protein, 11 aa, synthetic construct
  REGION 1..11: note = Synthetic peptide
SKPDNPGEDAP

SEQ ID NO: 44 - protein, 9 aa, synthetic construct
  REGION 1..9: note = Synthetic peptide
RESTENVPR

SEQ ID NO: 45 - protein, 9 aa, synthetic construct
  REGION 1..9: note = Synthetic peptide
ESTENVPRT

SEQ ID NO: 46 - protein, 12 aa, synthetic construct
  REGION 1..12: note = Synthetic peptide
SALRHYINLITR

SEQ ID NO: 47 - protein, 9 aa, synthetic construct
  REGION 1..9: note = Synthetic peptide
RYYSALRHY

SEQ ID NO: 48 - protein, 9 aa, synthetic construct
  REGION 1..9: note = Synthetic peptide
SALRHYINL

SEQ ID NO: 49 - protein, 8 aa, synthetic construct
  REGION 1..8: note = Synthetic peptide
HYINLITR

SEQ ID NO: 50 - protein, 11 aa, synthetic construct
  REGION 1..11: note = Synthetic peptide
YYSALRHYINL

SEQ ID NO: 51 - protein, 10 aa, synthetic construct
  REGION 1..10: note = Synthetic peptide
YSALRHYINL

SEQ ID NO: 52 - protein, 12 aa, synthetic construct
  REGION 1..12: note = Synthetic peptide
RYYSALRHYINL

SEQ ID NO: 53 - protein, 22 aa, synthetic construct
  REGION 1..22: note = Synthetic peptide
YPSKPDNPGEDAPAEDMARYYS

SEQ ID NO: 54 - protein, 12 aa, synthetic construct
  REGION 1..12: note = Synthetic peptide
SALRHYINLITR

SEQ ID NO: 55 - protein, 11 aa, synthetic construct
  REGION 1..11: note = Synthetic peptide
YPSKPDNPGED

SEQ ID NO: 56 - protein, 16 aa, synthetic construct
  REGION 1..16: note = Synthetic peptide
RESTENVPRTRLEDPA

SEQ ID NO: 57 - protein, 17 aa, synthetic construct
  REGION 1..17: note = Synthetic peptide
ESTENVPRTRLEDPAMW

SEQ ID NO: 58 - protein, 17 aa, synthetic construct
  REGION 1..17: note = Synthetic peptide
MRESTENVPRTRLEDPA

SEQ ID NO: 59 - protein, 13 aa, synthetic construct
  REGION 1..13: note = Synthetic peptide
RESTENVPRTRLE

SEQ ID NO: 60 - protein, 16 aa, synthetic construct
  REGION 1..16: note = Synthetic peptide
STENVPRTRLEDPAMW

SEQ ID NO: 61 - protein, 9 aa, synthetic construct
  REGION 1..9: note = Synthetic peptide
YPSKPDNPG

SEQ ID NO: 62 - protein, 21 aa, synthetic construct
  REGION 1..21: note = Synthetic peptide
SSPETLISDLLMRESTENVPR

SEQ ID NO: 63 - protein, 19 aa, synthetic construct
  REGION 1..19: note = Synthetic peptide
MRESTENVPRTRLEDPAMW

SEQ ID NO: 64 - protein, 12 aa, synthetic construct
  REGION 1..12: note = Synthetic peptide
ESTENVPRTRLE

SEQ ID NO: 65 - protein, 10 aa, synthetic construct
  REGION 1..10: note = Synthetic peptide
LRHYINLITR

SEQ ID NO: 66 - protein, 21 aa, synthetic construct
  REGION 1..21: note = Synthetic peptide
YPSKPDNPGEDAPAEDMARYY

SEQ ID NO: 67 - protein, 19 aa, synthetic construct
  REGION 1..19: note = Synthetic peptide
APAEDMARYYSALRHYINL

SEQ ID NO: 68 - protein, 20 aa, synthetic construct
  REGION 1..20: note = Synthetic peptide
YPSKPDNPGEDAPAEDMARY

SEQ ID NO: 69 - protein, 24 aa, synthetic construct
  REGION 1..24: note = Synthetic peptide
YPSKPDNPGEDAPAEDMARYYSAL

SEQ ID NO: 70 - protein, 14 aa, synthetic construct
  REGION 1..14: note = Synthetic peptide
YSALRHYINLITRQ

SEQ ID NO: 71 - protein, 18 aa, synthetic construct
  REGION 1..18: note = Synthetic peptide
APAEDMARYYSALRHYIN

SEQ ID NO: 72 - protein, 23 aa, synthetic construct
  REGION 1..23: note = Synthetic peptide
YPSKPDNPGEDAPAEDMARYYSA

SEQ ID NO: 73 - protein, 25 aa, synthetic construct
  REGION 1..25: note = Synthetic peptide
SKPDNPGEDAPAEDMARYYSALRHY

SEQ ID NO: 74 - protein, 16 aa, synthetic construct
  REGION 1..16: note = Synthetic peptide
LRHYINLITRQRYGKR

SEQ ID NO: 75 - protein, 14 aa, synthetic construct
  REGION 1..14: note = Synthetic peptide
DMARYYSALRHYIN

SEQ ID NO: 76 - protein, 15 aa, synthetic construct
  REGION 1..15: note = Synthetic peptide
DMARYYSALRHYINL

SEQ ID NO: 77 - protein, 17 aa, synthetic construct
  REGION 1..17: note = Synthetic peptide
AEDMARYYSALRHYINL

SEQ ID NO: 78 - protein, 13 aa, synthetic construct
  REGION 1..13: note = Synthetic peptide
ARYYSALRHYINL

SEQ ID NO: 79 - protein, 19 aa, synthetic construct
  REGION 1..19: note = Synthetic peptide
DMARYYSALRHYINLITRQ

SEQ ID NO: 80 - protein, 20 aa, synthetic construct
  REGION 1..20: note = Synthetic peptide
DAPAEDMARYYSALRHYINL

SEQ ID NO: 81 - protein, 16 aa, synthetic construct
  REGION 1..16: note = Synthetic peptide
AEDMARYYSALRHYIN

SEQ ID NO: 82 - protein, 23 aa, synthetic construct
  REGION 1..23: note = Synthetic peptide
SSPETLISDLLMRESTENVPRTR

SEQ ID NO: 83 - protein, 18 aa, synthetic construct
  REGION 1..18: note = Synthetic peptide
YPSKPDNPGEDAPAEDMA

SEQ ID NO: 84 - protein, 19 aa, synthetic construct
  REGION 1..19: note = Synthetic peptide
YPSKPDNPGEDAPAEDMAR

SEQ ID NO: 85 - protein, 11 aa, synthetic construct
  REGION 1..11: note = Synthetic peptide
YYSALRHYINL

SEQ ID NO: 86 - protein, 15 aa, synthetic construct
  REGION 1..15: note = Synthetic peptide
YPSKPDNPGEDAPAE

SEQ ID NO: 87 - protein, 16 aa, synthetic construct
  REGION 1..16: note = Synthetic peptide
YPSKPDNPGEDAPAED

SEQ ID NO: 88 - protein, 18 aa, synthetic construct
  REGION 1..18: note = Synthetic peptide
PAEDMARYYSALRHYINL

SEQ ID NO: 89 - protein, 16 aa, synthetic construct
  REGION 1..16: note = Synthetic peptide
EDMARYYSALRHYINL

SEQ ID NO: 90 - protein, 23 aa, synthetic construct
  REGION 1..23: note = Synthetic peptide
PGEDAPAEDMARYYSALRHYINL

SEQ ID NO: 91 - protein, 17 aa, synthetic construct
  REGION 1..17: note = Synthetic peptide
SSPETLISDLLMRESTE

SEQ ID NO: 92 - protein, 17 aa, synthetic construct
  REGION 1..17: note = Synthetic peptide
YPSKPDNPGEDAPAEDM

SEQ ID NO: 93 - protein, 11 aa, synthetic construct
  REGION 1..11: note = Synthetic peptide
SSPETLISDLL

SEQ ID NO: 94 - protein, 10 aa, synthetic construct
  REGION 1..10: note = Synthetic peptide
YSALRHYINL

SEQ ID NO: 95 - protein, 10 aa, synthetic construct
  REGION 1..10: note = Synthetic peptide
SPETLISDLL

SEQ ID NO: 96 - protein, 12 aa, synthetic construct
  REGION 1..12: note = Synthetic peptide
SSPETLISDLLM

SEQ ID NO: 97 - protein, 17 aa, synthetic construct
  REGION 1..17: note = Synthetic peptide
ARYYSALRHYINLITRQ

SEQ ID NO: 98 - protein, 11 aa, synthetic construct
  REGION 1..11: note = Synthetic peptide
LRHYINLITRQ

SEQ ID NO: 99 - protein, 14 aa, synthetic construct
  REGION 1..14: note = Synthetic peptide
LRHYINLITRQRYG

SEQ ID NO: 100 - protein, 22 aa, synthetic construct
  REGION 1..22: note = Synthetic peptide
SSPETLISDLLMRESTENVPRT

SEQ ID NO: 101 - protein, 14 aa, synthetic construct
  REGION 1..14: note = Synthetic peptide
YYSALRHYINLITR

SEQ ID NO: 102 - protein, 16 aa, synthetic construct
  REGION 1..16: note = Synthetic peptide
SALRHYINLITRQRYG

SEQ ID NO: 103 - protein, 25 aa, synthetic construct
  REGION 1..25: note = Synthetic peptide
SSPETLISDLLMRESTENVPRTRLE

SEQ ID NO: 104 - protein, 22 aa, synthetic construct
  REGION 1..22: note = Synthetic peptide
GEDAPAEDMARYYSALRHYINL

SEQ ID NO: 105 - protein, 14 aa, synthetic construct
  REGION 1..14: note = Synthetic peptide
YPSKPDNPGEDAPA

SEQ ID NO: 106 - protein, 16 aa, synthetic construct
  REGION 1..16: note = Synthetic peptide
YSALRHYINLITRQRY

SEQ ID NO: 107 - protein, 10 aa, synthetic construct
  REGION 1..10: note = Synthetic peptide
ARYYSALRHY

SEQ ID NO: 108 - protein, 10 aa, synthetic construct
  REGION 1..10: note = Synthetic peptide
YPSKPDNPGE

SEQ ID NO: 109 - protein, 13 aa, synthetic construct
  REGION 1..13: note = Synthetic peptide
YPSKPDNPGEDAP

SEQ ID NO: 110 - protein, 9 aa, synthetic construct
  REGION 1..9: note = Synthetic peptide
ESTENVPRT

SEQ ID NO: 111 - protein, 12 aa, synthetic construct
  REGION 1..12: note = Synthetic peptide
YPSKPDNPGEDA

SEQ ID NO: 112 - protein, 10 aa, synthetic construct
  REGION 1..10: note = Synthetic peptide
YYSALRHYIN

SEQ ID NO: 113 - protein, 13 aa, synthetic construct
  REGION 1..13: note = Synthetic peptide
SKPDNPGEDAPAE

SEQ ID NO: 114 - protein, 15 aa, synthetic construct
  REGION 1..15: note = Synthetic peptide
SALRHYINLITRQRY

SEQ ID NO: 115 - protein, 10 aa, synthetic construct
  REGION 1..10: note = Synthetic peptide
SSPETLISDL

SEQ ID NO: 116 - protein, 15 aa, synthetic construct
  REGION 1..15: note = Synthetic peptide
RYYSALRHYINLITR

SEQ ID NO: 117 - protein, 12 aa, synthetic construct
  REGION 1..12: note = Synthetic peptide
SALRHYINLITR

SEQ ID NO: 118 - protein, 19 aa, synthetic construct
  REGION 1..19: note = Synthetic peptide
APAEDMARYYSALRHYINL

SEQ ID NO: 119 - protein, 19 aa, synthetic construct
  REGION 1..19: note = Synthetic peptide
RYYSALRHYINLITRQRYG

SEQ ID NO: 120 - protein, 18 aa, synthetic construct
  REGION 1..18: note = Synthetic peptide
DMARYYSALRHYINLITR

SEQ ID NO: 121 - protein, 19 aa, synthetic construct
  REGION 1..19: note = Synthetic peptide
ARYYSALRHYINLITRQRY

SEQ ID NO: 122 - protein, 13 aa, synthetic construct
  REGION 1..13: note = Synthetic peptide
YSALRHYINLITR

SEQ ID NO: 123 - protein, 16 aa, synthetic construct
  REGION 1..16: note = Synthetic peptide
SALRHYINLITRQRYG

SEQ ID NO: 124 - protein, 18 aa, synthetic construct
  REGION 1..18: note = Synthetic peptide
RYYSALRHYINLITRQRY

SEQ ID NO: 125 - protein, 14 aa, synthetic construct
  REGION 1..14: note = Synthetic peptide
SALRHYINLITRQR

SEQ ID NO: 126 - protein, 23 aa, synthetic construct
  REGION 1..23: note = Synthetic peptide
APAEDMARYYSALRHYINLITRQ

SEQ ID NO: 127 - protein, 15 aa, synthetic construct
  REGION 1..15: note = Synthetic peptide
SALRHYINLITRQRY

SEQ ID NO: 128 - protein, 14 aa, synthetic construct
  REGION 1..14: note = Synthetic peptide
YYSALRHYINLITR

SEQ ID NO: 129 - protein, 22 aa, synthetic construct
  REGION 1..22: note = Synthetic peptide
DMARYYSALRHYINLITRQRYG

SEQ ID NO: 130 - protein, 19 aa, synthetic construct
  REGION 1..19: note = Synthetic peptide
DMARYYSALRHYINLITRQ

SEQ ID NO: 131 - protein, 21 aa, synthetic construct
  REGION 1..21: note = Synthetic peptide
AEDMARYYSALRHYINLITRQ

SEQ ID NO: 132 - protein, 18 aa, synthetic construct
  REGION 1..18: note = Synthetic peptide
YYSALRHYINLITRQRYG

SEQ ID NO: 133 - protein, 15 aa, synthetic construct
  REGION 1..15: note = Synthetic peptide
ALRHYINLITRQRYG

SEQ ID NO: 134 - protein, 12 aa, synthetic construct
  REGION 1..12: note = Synthetic peptide
SSPETLISDLLM

SEQ ID NO: 135 - protein, 21 aa, synthetic construct
  REGION 1..21: note = Synthetic peptide
APAEDMARYYSALRHYINLIT

SEQ ID NO: 136 - protein, 16 aa, synthetic construct
  REGION 1..16: note = Synthetic peptide
ARYYSALRHYINLITR

SEQ ID NO: 137 - protein, 20 aa, synthetic construct
  REGION 1..20: note = Synthetic peptide
DMARYYSALRHYINLITRQR

SEQ ID NO: 138 - protein, 22 aa, synthetic construct
  REGION 1..22: note = Synthetic peptide
APAEDMARYYSALRHYINLITR

SEQ ID NO: 139 - protein, 17 aa, synthetic construct
  REGION 1..17: note = Synthetic peptide
RYYSALRHYINLITRQR

SEQ ID NO: 140 - protein, 24 aa, synthetic construct
  REGION 1..24: note = Synthetic peptide
AEDMARYYSALRHYINLITRQRYG

SEQ ID NO: 141 - protein, 15 aa, synthetic construct
  REGION 1..15: note = Synthetic peptide
DMARYYSALRHYINL

SEQ ID NO: 142 - protein, 20 aa, synthetic construct
  REGION 1..20: note = Synthetic peptide
APAEDMARYYSALRHYINLI

SEQ ID NO: 143 - protein, 20 aa, synthetic construct
  REGION 1..20: note = Synthetic peptide
AEDMARYYSALRHYINLITR

SEQ ID NO: 144 - protein, 24 aa, synthetic construct
  REGION 1..24: note = Synthetic peptide
APAEDMARYYSALRHYINLITRQR

SEQ ID NO: 145 - protein, 13 aa, synthetic construct
  REGION 1..13: note = Synthetic peptide
YYSALRHYINLIT

SEQ ID NO: 146 - protein, 25 aa, synthetic construct
  REGION 1..25: note = Synthetic peptide
APAEDMARYYSALRHYINLITRQRY

SEQ ID NO: 147 - protein, 20 aa, synthetic construct
  REGION 1..20: note = Synthetic peptide
ARYYSALRHYINLITRQRYG

SEQ ID NO: 148 - protein, 14 aa, synthetic construct
  REGION 1..14: note = Synthetic peptide
ALRHYINLITRQRY

SEQ ID NO: 149 - protein, 16 aa, synthetic construct
  REGION 1..16: note = Synthetic peptide
YSALRHYINLITRQRY

SEQ ID NO: 150 - protein, 11 aa, synthetic construct
  REGION 1..11: note = Synthetic peptide
SPETLISDLLM

SEQ ID NO: 151 - protein, 12 aa, synthetic construct
  REGION 1..12: note = Synthetic peptide
RYYSALRHYINL

SEQ ID NO: 152 - protein, 16 aa, synthetic construct
  REGION 1..16: note = Synthetic peptide
YYSALRHYINLITRQR

SEQ ID NO: 153 - protein, 11 aa, synthetic construct
  REGION 1..11: note = Synthetic peptide
SSPETLISDLL

SEQ ID NO: 154 - protein, 10 aa, synthetic construct
  REGION 1..10: note = Synthetic peptide
SPETLISDLL

SEQ ID NO: 155 - protein, 21 aa, synthetic construct
  REGION 1..21: note = Synthetic peptide
SSPETLISDLLMRESTENVPR

SEQ ID NO: 156 - protein, 13 aa, synthetic construct
  REGION 1..13: note = Synthetic peptide
SALRHYINLITRQ

SEQ ID NO: 157 - protein, 24 aa, synthetic construct
  REGION 1..24: note = Synthetic peptide
ISDLLMRESTENVPRTRLEDPAMW

SEQ ID NO: 158 - protein, 17 aa, synthetic construct
  REGION 1..17: note = Synthetic peptide
YYSALRHYINLITRQRY

SEQ ID NO: 159 - protein, 25 aa, synthetic construct
  REGION 1..25: note = Synthetic peptide
DMARYYSALRHYINLITRQRYGKRS

SEQ ID NO: 160 - protein, 14 aa, synthetic construct
  REGION 1..14: note = Synthetic peptide
RYYSALRHYINLIT

SEQ ID NO: 161 - protein, 23 aa, synthetic construct
  REGION 1..23: note = Synthetic peptide
AEDMARYYSALRHYINLITRQRY

SEQ ID NO: 162 - protein, 10 aa, synthetic construct
  REGION 1..10: note = Synthetic peptide
PSKPDNPGED

SEQ ID NO: 163 - protein, 10 aa, synthetic construct
  REGION 1..10: note = Synthetic peptide
VILKKATEYV

SEQ ID NO: 164 - protein, 9 aa, synthetic construct
  REGION 1..9: note = Synthetic peptide
GADGVGKSA